European Patent Application EP 4 410 837 A1, published August 7, 2024. Title: 抗LAG3双特异性抗体、药物组合物及用途. Applicant: 中山康方生物医药有限公司. The sequence listing filed with the application follows.

SEQUENCE LISTING (48 sequences)

SEQ ID NO: 1 - DNA, 360 bp, synthetic construct
  source 1..360: mol_type = other DNA
caggtgcagctgcagcagtggggagctggactgctgaaacctagcgagacactgagcctgacctgtgctgtgtacggcggatctatcagcgattactactggaactggatcaggcagccccctggaaagggactggaatggatcggagagatcaaccacaggggcaccaccaactccaatccctctctgaagagcagggtgacactgagcctcgacacaagcaagaatcagttcagcctgaagctgaggtccgtgaccgctgctgatacagctgtgtactactgtgccttcggctacagcgattacgagtacgattggttcgacccttggggccagggaacactggttacagtgagctcc

SEQ ID NO: 2 - protein, 120 aa, synthetic construct
QVQLQQWGAGLLKPSETLSLTCAVYGGSISDYYWNWIRQPPGKGLEWIGEINHRGTTNSNPSLKSRVTLSLDTSKNQFSLKLRSVTAADTAVYYCAFGYSDYEYDWFDPWGQGTLVTVSS

SEQ ID NO: 3 - DNA, 321 bp, synthetic construct
  source 1..321: mol_type = other DNA
gagatcgttctgacccagagcccagctacactgagcctgtctcctggagagagggctacactgtcctgcagagctagccagaccatcagcagctacctggcttggtaccagcagaagcctggccaagctccaaggctgctgatctacgacgcctctaatagggccaccggcatccctgctagattctctggaagcggcagcggaaccgactttacactgacaatcagctccctggagcccgaggatttcgctgtttactactgtcagcagcgcagcaactggcccatcacattcggacagggcacaaatctggagatcaag

SEQ ID NO: 4 - protein, 107 aa, synthetic construct
EIVLTQSPATLSLSPGERATLSCRASQTISSYLAWYQQKPGQAPRLLIYDASNRATGIPARFSGSGSGTDFTLTISSLEPEDFAVYYCQQRSNWPITFGQGTNLEIK

SEQ ID NO: 5 - protein, 8 aa, synthetic construct
GGSISDYY

SEQ ID NO: 6 - protein, 7 aa, synthetic construct
INHRGTT

SEQ ID NO: 7 - protein, 14 aa, synthetic construct
AFGYSDYEYDWFDP

SEQ ID NO: 8 - protein, 6 aa, synthetic construct
QTISSY

SEQ ID NO: 9 - skipped

SEQ ID NO: 10 - protein, 9 aa, synthetic construct
QQRSNWPIT

SEQ ID NO: 11 - protein, 450 aa, synthetic construct
QVQLQQWGAGLLKPSETLSLTCAVYGGSISDYYWNWIRQPPGKGLEWIGEINHRGTTNSNPSLKSRVTLSLDTSKNQFSLKLRSVTAADTAVYYCAFGYSDYEYDWFDPWGQGTLVTVSSASTKGPSVFPLAPSSKSTSGGTAALGCLVKDYFPEPVTVSWNSGALTSGVHTFPAVLQSSGLYSLSSVVTVPSSSLGTQTYICNVNHKPSNTKVDKKVEPKSCDKTHTCPPCPAPEAAGAPSVFLFPPKPKDTLMISRTPEVTCVVVDVSHEDPEVKFNWYVDGVEVHNAKTKPREEQYNSTYRVVSVLTVLHQDWLNGKEYKCKVSNKALPAPIEKTISKAKGQPREPQVYTLPPSRDELTKNQVSLTCLVKGFYPSDIAVEWESNGQPENNYKTTPPVLDSDGSFFLYSKLTVDKSRWQQGNVFSCSVMHEALHNHYTQKSLSLSPGK

SEQ ID NO: 12 - protein, 214 aa, synthetic construct
EIVLTQSPATLSLSPGERATLSCRASQTISSYLAWYQQKPGQAPRLLIYDASNRATGIPARFSGSGSGTDFTLTISSLEPEDFAVYYCQQRSNWPITFGQGTNLEIKRTVAAPSVFIFPPSDEQLKSGTASVVCLLNNFYPREAKVQWKVDNALQSGNSQESVTEQDSKDSTYSLSSTLTLSKADYEKHKVYACEVTHQGLSSPVTKSFNRGEC

SEQ ID NO: 13 - protein, 447 aa, synthetic construct
QVQLQQWGAGLLKPSETLSLTCAVYGGSISDYYWNWIRQPPGKGLEWIGEINHRGTTNSNPSLKSRVTLSLDTSKNQFSLKLRSVTAADTAVYYCAFGYSDYEYDWFDPWGQGTLVTVSSASTKGPSVFPLAPCSRSTSESTAALGCLVKDYFPEPVTVSWNSGALTSGVHTFPAVLQSSGLYSLSSVVTVPSSSLGTKTYTCNVDHKPSNTKVDKRVESKYGPPCPPCPAPEAAGGPSVFLFPPKPKDTLMISRTPEVTCVVVDVSQEDPEVQFNWYVDGVEVHNAKTKPREEQFNSTYRVVSVLTVLHQDWLNGKEYKCKVSNKGLPSSIEKTISKAKGQPREPQVYTLPPSQEEMTKNQVSLTCLVKGFYPSDIAVEWESNGQPENNYKTTPPVLDSDGSFFLYSRLTVDKSRWQEGNVFSCSVMHEALHNHYTQKSLSLSLGK

SEQ ID NO: 14 - DNA, 354 bp, synthetic construct
  source 1..354: mol_type = other DNA
gaggtcaaactggtggagagcggcggcgggctggtgaagcccggcgggtcactgaaactgagctgcgccgcttccggcttcgcctttagctcctacgacatgtcatgggtgaggcagacccctgagaagcgcctggaatgggtcgctactatcagcggaggcgggcgatacacctactatcctgactctgtcaaagggagattcacaattagtcgggataacgccagaaatactctgtatctgcagatgtctagtctgcggtccgaggatacagctctgtactattgtgcaaaccggtacggcgaagcatggtttgcctattggggacagggcaccctggtgacagtctctgcc

SEQ ID NO: 15 - protein, 118 aa, synthetic construct
EVKLVESGGGLVKPGGSLKLSCAASGFAFSSYDMSWVRQTPEKRLEWVATISGGGRYTYYPDSVKGRFTISRDNARNTLYLQMSSLRSEDTALYYCANRYGEAWFAYWGQGTLVTVSA

SEQ ID NO: 16 - DNA, 321 bp, synthetic construct
  source 1..321: mol_type = other DNA
gacattaagatgacacagtccccttcctcaatgtacgctagcctgggcgagcgagtgaccttcacatgcaaagcatcccaggacatcaacacatacctgtcttggtttcagcagaagccaggcaaaagccccaagaccctgatctaccgggccaatagactggtggacggggtccccagcagattctccggatctggcagtgggcaggattactccctgaccatcagctccctggagtatgaagacatgggcatctactattgcctgcagtatgatgagttccctctgacctttggagcaggcacaaaactggaactgaag

SEQ ID NO: 17 - protein, 107 aa, synthetic construct
DIKMTQSPSSMYASLGERVTFTCKASQDINTYLSWFQQKPGKSPKTLIYRANRLVDGVPSRFSGSGSGQDYSLTISSLEYEDMGIYYCLQYDEFPLTFGAGTKLELK

SEQ ID NO: 18 - DNA, 354 bp, synthetic construct
  source 1..354: mol_type = other DNA
gaagtgcagctggtcgagtctgggggagggctggtgcagcccggcgggtcactgcgactgagctgcgcagcttccggattcgcctttagctcctacgacatgtcctgggtgcgacaggcaccaggaaagggactggattgggtcgctactatctcaggaggcgggagatacacctactatcctgacagcgtcaagggccggttcacaatctctagagataacagtaagaacaatctgtatctgcagatgaacagcctgagggctgaggacaccgcactgtactattgtgccaaccgctacggggaagcatggtttgcctattgggggcagggaaccctggtgacagtctctagt

SEQ ID NO: 19 - protein, 118 aa, synthetic construct
EVQLVESGGGLVQPGGSLRLSCAASGFAFSSYDMSWVRQAPGKGLDWVATISGGGRYTYYPDSVKGRFTISRDNSKNNLYLQMNSLRAEDTALYYCANRYGEAWFAYWGQGTLVTVSS

SEQ ID NO: 20 - DNA, 321 bp, synthetic construct
  source 1..321: mol_type = other DNA
gacattcagatgactcagagcccctcctccatgtccgcctctgtgggcgacagggtcaccttcacatgccgcgctagtcaggatatcaacacctacctgagctggtttcagcagaagccagggaaaagccccaagacactgatctaccgggctaatagactggtgtctggagtcccaagtcggttcagtggctcagggagcggacaggactacactctgaccatcagctccctgcagcctgaggacatggcaacctactattgcctgcagtatgatgagttcccactgacctttggcgccgggacaaaactggagctgaag

SEQ ID NO: 21 - protein, 107 aa, synthetic construct
DIQMTQSPSSMSASVGDRVTFTCRASQDINTYLSWFQQKPGKSPKTLIYRANRLVSGVPSRFSGSGSGQDYTLTISSLQPEDMATYYCLQYDEFPLTFGAGTKLELK

SEQ ID NO: 22 - DNA, 1344 bp, synthetic construct
  source 1..1344: mol_type = other DNA
gaagtgcagctggtcgagtctgggggagggctggtgcagcccggcgggtcactgcgactgagctgcgcagcttccggattcgcctttagctcctacgacatgtcctgggtgcgacaggcaccaggaaagggactggattgggtcgctactatctcaggaggcgggagatacacctactatcctgacagcgtcaagggccggttcacaatctctagagataacagtaagaacaatctgtatctgcagatgaacagcctgagggctgaggacaccgcactgtactattgtgccaaccgctacggggaagcatggtttgcctattgggggcagggaaccctggtgacagtctctagtgccagcaccaaaggacctagcgtgtttcctctcgccccctcctccaaaagcaccagcggaggaaccgctgctctcggatgtctggtgaaggactacttccctgaacccgtcaccgtgagctggaatagcggcgctctgacaagcggagtccatacattccctgctgtgctgcaaagcagcggactctattccctgtccagcgtcgtcacagtgcccagcagcagcctgggcacccagacctacatctgtaacgtcaaccacaagccctccaacaccaaggtggacaagaaagtggagcccaaatcctgcgacaagacacacacctgtcccccctgtcctgctcccgaactcctcggaggccctagcgtcttcctctttcctcccaaacccaaggacaccctcatgatcagcagaacccctgaagtcacctgtgtcgtcgtggatgtcagccatgaggaccccgaggtgaaattcaactggtatgtcgatggcgtcgaggtgcacaacgccaaaaccaagcccagggaggaacagtacaactccacctacagggtggtgtccgtgctgacagtcctccaccaggactggctgaacggcaaggagtacaagtgcaaggtgtccaacaaggctctccctgcccccattgagaagaccatcagcaaggccaaaggccaacccagggagccccaggtctatacactgcctccctccagggacgaactcaccaagaaccaggtgtccctgacctgcctggtcaagggcttttatcccagcgacatcgccgtcgagtgggagtccaacggacagcccgagaataactacaagaccacccctcctgtcctcgactccgacggctccttcttcctgtacagcaagctgaccgtggacaaaagcaggtggcagcagggaaacgtgttctcctgcagcgtgatgcacgaagccctccacaaccactacacccagaaaagcctgtccctgagccccggcaaa

SEQ ID NO: 23 - protein, 448 aa, synthetic construct
EVQLVESGGGLVQPGGSLRLSCAASGFAFSSYDMSWVRQAPGKGLDWVATISGGGRYTYYPDSVKGRFTISRDNSKNNLYLQMNSLRAEDTALYYCANRYGEAWFAYWGQGTLVTVSSASTKGPSVFPLAPSSKSTSGGTAALGCLVKDYFPEPVTVSWNSGALTSGVHTFPAVLQSSGLYSLSSVVTVPSSSLGTQTYICNVNHKPSNTKVDKKVEPKSCDKTHTCPPCPAPELLGGPSVFLFPPKPKDTLMISRTPEVTCVVVDVSHEDPEVKFNWYVDGVEVHNAKTKPREEQYNSTYRVVSVLTVLHQDWLNGKEYKCKVSNKALPAPIEKTISKAKGQPREPQVYTLPPSRDELTKNQVSLTCLVKGFYPSDIAVEWESNGQPENNYKTTPPVLDSDGSFFLYSKLTVDKSRWQQGNVFSCSVMHEALHNHYTQKSLSLSPGK

SEQ ID NO: 24 - DNA, 642 bp, synthetic construct
  source 1..642: mol_type = other DNA
gacattcagatgactcagagcccctcctccatgtccgcctctgtgggcgacagggtcaccttcacatgccgcgctagtcaggatatcaacacctacctgagctggtttcagcagaagccagggaaaagccccaagacactgatctaccgggctaatagactggtgtctggagtcccaagtcggttcagtggctcagggagcggacaggactacactctgaccatcagctccctgcagcctgaggacatggcaacctactattgcctgcagtatgatgagttcccactgacctttggcgccgggacaaaactggagctgaagcgaactgtggccgctccctccgtcttcatttttcccccttctgacgaacagctgaaatcaggcacagccagcgtggtctgtctgctgaacaatttctaccctagagaggcaaaagtgcagtggaaggtcgataacgccctgcagtccggcaacagccaggagagtgtgactgaacaggactcaaaagatagcacctattccctgtctagtacactgactctgtccaaggctgattacgagaagcacaaagtgtatgcatgcgaagtgacacatcagggactgtcaagccccgtgactaagtcttttaaccggggcgaatgt

SEQ ID NO: 25 - protein, 214 aa, synthetic construct
DIQMTQSPSSMSASVGDRVTFTCRASQDINTYLSWFQQKPGKSPKTLIYRANRLVSGVPSRFSGSGSGQDYTLTISSLQPEDMATYYCLQYDEFPLTFGAGTKLELKRTVAAPSVFIFPPSDEQLKSGTASVVCLLNNFYPREAKVQWKVDNALQSGNSQESVTEQDSKDSTYSLSSTLTLSKADYEKHKVYACEVTHQGLSSPVTKSFNRGEC

SEQ ID NO: 26 - protein, 8 aa, synthetic construct
GFAFSSYD

SEQ ID NO: 27 - protein, 8 aa, synthetic construct
ISGGGRYT

SEQ ID NO: 28 - protein, 11 aa, synthetic construct
ANRYGEAWFAY

SEQ ID NO: 29 - protein, 6 aa, synthetic construct
QDINTY

SEQ ID NO: 30 - skipped

SEQ ID NO: 31 - protein, 9 aa, synthetic construct
LQYDEFPLT

SEQ ID NO: 32 - protein, 445 aa, synthetic construct
EVQLVESGGGLVQPGGSLRLSCAASGFAFSSYDMSWVRQAPGKGLDWVATISGGGRYTYYPDSVKGRFTISRDNSKNNLYLQMNSLRAEDTALYYCANRYGEAWFAYWGQGTLVTVSSASTKGPSVFPLAPCSRSTSESTAALGCLVKDYFPEPVTVSWNSGALTSGVHTFPAVLQSSGLYSLSSVVTVPSSSLGTKTYTCNVDHKPSNTKVDKRVESKYGPPCPPCPAPEAAGGPSVFLFPPKPKDTLMISRTPEVTCVVVDVSQEDPEVQFNWYVDGVEVHNAKTKPREEQFNSTYRVVSVLTVLHQDWLNGKEYKCKVSNKGLPSSIEKTISKAKGQPREPQVYTLPPSQEEMTKNQVSLTCLVKGFYPSDIAVEWESNGQPENNYKTTPPVLDSDGSFFLYSRLTVDKSRWQEGNVFSCSVMHEALHNHYTQKSLSLSLGK

SEQ ID NO: 33 - DNA, 1344 bp, synthetic construct
  source 1..1344: mol_type = other DNA
gaagtgcagctggtcgagtctgggggagggctggtgcagcccggcgggtcactgcgactgagctgcgcagcttccggattcgcctttagctcctacgacatgtcctgggtgcgacaggcaccaggaaagggactggattgggtcgctactatctcaggaggcgggagatacacctactatcctgacagcgtcaagggccggttcacaatctctagagataacagtaagaacaatctgtatctgcagatgaacagcctgagggctgaggacaccgcactgtactattgtgccaaccgctacggggaagcatggtttgcctattgggggcagggaaccctggtgacagtctctagtgccagcaccaaagggcccagcgtgtttcctctcgccccctcctccaaaagcaccagcggaggaaccgctgctctcggatgtctggtgaaggactacttccctgaacccgtcaccgtgagctggaatagcggcgctctgacaagcggagtccatacattccctgctgtgctgcaaagcagcggactctattccctgtccagcgtcgtcacagtgcccagcagcagcctgggcacccagacctacatctgtaacgtcaaccacaagccctccaacaccaaggtggacaagaaagtggagcccaaatcctgcgacaagacacacacctgtcccccctgtcctgctcccgaagctgctggagcccctagcgtcttcctctttcctcccaaacccaaggacaccctcatgatcagcagaacccctgaagtcacctgtgtcgtcgtggatgtcagccatgaggaccccgaggtgaaattcaactggtatgtcgatggcgtcgaggtgcacaacgccaaaaccaagcccagggaggaacagtacaactccacctacagggtggtgtccgtgctgacagtcctccaccaggactggctgaacggcaaggagtacaagtgcaaggtgtccaacaaggctctccctgcccccattgagaagaccatcagcaaggccaaaggccaacccagggagccccaggtctatacactgcctccctccagggacgaactcaccaagaaccaggtgtccctgacctgcctggtcaagggcttttatcccagcgacatcgccgtcgagtgggagtccaacggacagcccgagaataactacaagaccacccctcctgtcctcgactccgacggctccttcttcctgtacagcaagctgaccgtggacaaaagcaggtggcagcagggaaacgtgttctcctgcagcgtgatgcacgaagccctccacaaccactacacccagaaaagcctgtccctgagccccggcaaa

SEQ ID NO: 34 - protein, 448 aa, synthetic construct
EVQLVESGGGLVQPGGSLRLSCAASGFAFSSYDMSWVRQAPGKGLDWVATISGGGRYTYYPDSVKGRFTISRDNSKNNLYLQMNSLRAEDTALYYCANRYGEAWFAYWGQGTLVTVSSASTKGPSVFPLAPSSKSTSGGTAALGCLVKDYFPEPVTVSWNSGALTSGVHTFPAVLQSSGLYSLSSVVTVPSSSLGTQTYICNVNHKPSNTKVDKKVEPKSCDKTHTCPPCPAPEAAGAPSVFLFPPKPKDTLMISRTPEVTCVVVDVSHEDPEVKFNWYVDGVEVHNAKTKPREEQYNSTYRVVSVLTVLHQDWLNGKEYKCKVSNKALPAPIEKTISKAKGQPREPQVYTLPPSRDELTKNQVSLTCLVKGFYPSDIAVEWESNGQPENNYKTTPPVLDSDGSFFLYSKLTVDKSRWQQGNVFSCSVMHEALHNHYTQKSLSLSPGK

SEQ ID NO: 35 - protein, 15 aa, synthetic construct
GGGGSGGGGSGGGGS

SEQ ID NO: 36 - protein, 20 aa, synthetic construct
GGGGSGGGGSGGGGSGGGGS

SEQ ID NO: 37 - protein, 21 aa, synthetic construct
GGGGSGGGGSGGGGSGGGGSG

SEQ ID NO: 38 - protein, 108 aa, synthetic construct
DIQMTQSPSSMSASVGDRVTFTCRASQDINTYLSWFQQKPGKSPKTLIYRANRLVSGVPSRFSGSGSGQDYTLTISSLQPEDMATYYCLQYDEFPLTFGAGTKLELKR

SEQ ID NO: 39 - protein, 330 aa, synthetic construct [sequence omitted]

SEQ ID NO: 40 - protein, 107 aa, synthetic construct [sequence omitted]

SEQ ID NO: 41 - DNA, 321 bp, synthetic construct
  source 1..321: mol_type = other DNA
gagatcgttctgacccagagcccagctacactgagcctgtctcctggagagagggctacactgtcctgcagagctagccagaccatcagcagctacctggcttggtaccagcagaagcctggccaagctccaaggctgctgatctacgacggctctaatagggccaccggcatccctgctagattctctggaagcggcagcggaaccgactttacactgacaatcagctccctggagcccgaggatttcgctgtttactactgtcagcagcgcagcaactggcccctcacattcggacagggcacaaatctggagatcaag

SEQ ID NO: 42 - protein, 107 aa, synthetic construct
EIVLTQSPATLSLSPGERATLSCRASQTISSYLAWYQQKPGQAPRLLIYDGSNRATGIPARFSGSGSGTDFTLTISSLEPEDFAVYYCQQRSNWPLTFGQGTNLEIK

SEQ ID NO: 43 - DNA, 321 bp, synthetic construct
  source 1..321: mol_type = other DNA
gagatcgttctgacccagagcccagctacactgagcctgtctcctggagagagggctacactgtcctgcagagctagccagtccatcagcagctacctggcttggtaccagcagaagcctggccaagctccaaggctgctgatctacgacggctctaatagggccaccggcatccctgctagattctctggaagcggcagcggaaccgactttacactgacaatcagctccctggagcccgaggatttcgctgtttactactgtcagcagcgcagcaactggcccatcacattcggacagggcacaaatctggagatcaag

SEQ ID NO: 44 - protein, 107 aa, synthetic construct
EIVLTQSPATLSLSPGERATLSCRASQSISSYLAWYQQKPGQAPRLLIYDGSNRATGIPARFSGSGSGTDFTLTISSLEPEDFAVYYCQQRSNWPITFGQGTNLEIK

SEQ ID NO: 45 - protein, 327 aa, synthetic construct
ASTKGPSVFPLAPCSRSTSESTAALGCLVKDYFPEPVTVSWNSGALTSGVHTFPAVLQSSGLYSLSSVVTVPSSSLGTKTYTCNVDHKPSNTKVDKRVESKYGPPCPPCPAPEFLGGPSVFLFPPKPKDTLMISRTPEVTCVVVDVSQEDPEVQFNWYVDGVEVHNAKTKPREEQFNSTYRVVSVLTVLHQDWLNGKEYKCKVSNKGLPSSIEKTISKAKGQPREPQVYTLPPSQEEMTKNQVSLTCLVKGFYPSDIAVEWESNGQPENNYKTTPPVLDSDGSFFLYSRLTVDKSRWQEGNVFSCSVMHEALHNHYTQKSLSLSLGK

SEQ ID NO: 46 - skipped

SEQ ID NO: 47 - protein, 9 aa, synthetic construct
QQRSNWPLT

SEQ ID NO: 48 - protein, 6 aa, synthetic construct
QSISSY